European Patent Specification EP 3 587 589 B1, published September 13, 2023. Title: REAGENTS AND METHODS FOR THE ANALYSIS OF CIRCULATING MICROPARTICLES. Applicant: CS Genetics Limited. The sequence listing filed with the application follows.

SEQUENCE LISTING (303 sequences)

SEQ ID NO: 1 - DNA, 38 bp, Artificial Sequence
  Primer
ctcgatgctacgtgactactgcgtcgaggagtctatcc

SEQ ID NO: 2 - DNA, 96 bp, Artificial Sequence
  Primer
atacctgactgctcgtcagttgagcgaattccgtatgggtagcaaggtccaagagaggctccatcctcactcgcctgactacgacaagacctactg

SEQ ID NO: 3 - DNA, 98 bp, Artificial Sequence
  Primer
tccagtaggtcttgtcgtagtcaggcgagtgaggatggagcctctcttggaccttgctacccatacggaattcgctcaactgacgagcagtcaggtat

SEQ ID NO: 4 - DNA, 22 bp, Artificial Sequence
  Primer
ctcgatgctacgtgactactgc

SEQ ID NO: 5 - DNA, 22 bp, Artificial Sequence
  Primer
cagtaggtcttgtcgtagtcag

SEQ ID NO: 6 - DNA, 45 bp, Artificial Sequence
  Primer
atggtacacacctacactactcggacgctcttccgatcttgacct

SEQ ID NO: 7 - DNA, 44 bp, Artificial Sequence
  Primer
aggtcaagatcggaagagcgtccgagtagtgtaggtgtgtacca

SEQ ID NO: 8 - DNA, 22 bp, Artificial Sequence
  Primer
tggtacacacctacactactcg

SEQ ID NO: 9 - DNA, 20 bp, Artificial Sequence
  Primer
ccatacggaattcgctcaac

SEQ ID NO: 10 - DNA, 42 bp, Artificial Sequence
  Primer
gttgagcgaattccgtatggtggtacacacctacactactcg

SEQ ID NO: 11 - DNA, 46 bp, Artificial Sequence
  Primer
taggacgatacgagtgtgtactcgtggtacacacctacactactcg

SEQ ID NO: 12 - DNA, 42 bp, Artificial Sequence
  Primer
cgagtagtgtaggtgtgtaccaccatacggaattcgctcaac

SEQ ID NO: 13 - DNA, 44 bp, Artificial Sequence
  Primer
ctgtcaaggtagactagcatgctcccatacggaattcgctcaac

SEQ ID NO: 14 - DNA, 24 bp, Artificial Sequence
  Primer
taggacgatacgagtgtgtactcg

SEQ ID NO: 15 - DNA, 24 bp, Artificial Sequence
  Primer
ctgtcaaggtagactagcatgctc

SEQ ID NO: 16 - DNA, 56 bp, Artificial Sequence
  Primer
ctcggcattcctgctgaaccgctcttccgatctgctcaactgacgagcagtcaggt

SEQ ID NO: 17 - DNA, 39 bp, Artificial Sequence
  Primer
acactctttccctacacgacgctcttccgatcttgacct

SEQ ID NO: 18 - DNA, 20 bp, Artificial Sequence
  Sequence used in the synthesis of sub-barcode molecule library
aaacggatagactcctcgac

SEQ ID NO: 19 - DNA, 20 bp, Artificial Sequence
  Sequence used in the synthesis of sub-barcode molecule library
aaagggatagactcctcgac

SEQ ID NO: 20 - DNA, 20 bp, Artificial Sequence
  Sequence used in the synthesis of sub-barcode molecule library
aaatggatagactcctcgac

SEQ ID NO: 21 - DNA, 20 bp, Artificial Sequence
  Sequence used in the synthesis of sub-barcode molecule library
aacaggatagactcctcgac

SEQ ID NO: 22 - DNA, 20 bp, Artificial Sequence
  Sequence used in the synthesis of sub-barcode molecule library
aaccggatagactcctcgac

SEQ ID NO: 23 - DNA, 20 bp, Artificial Sequence
  Sequence used in the synthesis of sub-barcode molecule library
aacgggatagactcctcgac

SEQ ID NO: 24 - DNA, 20 bp, Artificial Sequence
  Sequence used in the synthesis of sub-barcode molecule library
aactggatagactcctcgac

SEQ ID NO: 25 - DNA, 20 bp, Artificial Sequence
  Sequence used in the synthesis of sub-barcode molecule library
aagaggatagactcctcgac

SEQ ID NO: 26 - DNA, 20 bp, Artificial Sequence
  Sequence used in the synthesis of sub-barcode molecule library
aagcggatagactcctcgac

SEQ ID NO: 27 - DNA, 20 bp, Artificial Sequence
  Sequence used in the synthesis of sub-barcode molecule library
aaggggatagactcctcgac

SEQ ID NO: 28 - DNA, 20 bp, Artificial Sequence
  Sequence used in the synthesis of sub-barcode molecule library
aagtggatagactcctcgac

SEQ ID NO: 29 - DNA, 20 bp, Artificial Sequence
  Sequence used in the synthesis of sub-barcode molecule library
aataggatagactcctcgac

SEQ ID NO: 30 - DNA, 20 bp, Artificial Sequence
  Sequence used in the synthesis of sub-barcode molecule library
aatcggatagactcctcgac

SEQ ID NO: 31 - DNA, 20 bp, Artificial Sequence
  Sequence used in the synthesis of sub-barcode molecule library
aatgggatagactcctcgac

SEQ ID NO: 32 - DNA, 20 bp, Artificial Sequence
  Sequence used in the synthesis of sub-barcode molecule library
aattggatagactcctcgac

SEQ ID NO: 33 - DNA, 20 bp, Artificial Sequence
  Sequence used in the synthesis of sub-barcode molecule library
acaaggatagactcctcgac

SEQ ID NO: 34 - DNA, 20 bp, Artificial Sequence
  Sequence used in the synthesis of sub-barcode molecule library
acacggatagactcctcgac

SEQ ID NO: 35 - DNA, 20 bp, Artificial Sequence
  Sequence used in the synthesis of sub-barcode molecule library
acagggatagactcctcgac

SEQ ID NO: 36 - DNA, 20 bp, Artificial Sequence
  Sequence used in the synthesis of sub-barcode molecule library
acatggatagactcctcgac

SEQ ID NO: 37 - DNA, 20 bp, Artificial Sequence
  Sequence used in the synthesis of sub-barcode molecule library
accaggatagactcctcgac

SEQ ID NO: 38 - DNA, 20 bp, Artificial Sequence
  Sequence used in the synthesis of sub-barcode molecule library
acccggatagactcctcgac

SEQ ID NO: 39 - DNA, 20 bp, Artificial Sequence
  Sequence used in the synthesis of sub-barcode molecule library
accgggatagactcctcgac

SEQ ID NO: 40 - DNA, 20 bp, Artificial Sequence
  Sequence used in the synthesis of sub-barcode molecule library
acctggatagactcctcgac

SEQ ID NO: 41 - DNA, 20 bp, Artificial Sequence
  Sequence used in the synthesis of sub-barcode molecule library
acgaggatagactcctcgac

SEQ ID NO: 42 - DNA, 20 bp, Artificial Sequence
  Sequence used in the synthesis of sub-barcode molecule library
acgcggatagactcctcgac

SEQ ID NO: 43 - DNA, 20 bp, Artificial Sequence
  Sequence used in the synthesis of sub-barcode molecule library
acggggatagactcctcgac

SEQ ID NO: 44 - DNA, 20 bp, Artificial Sequence
  Sequence used in the synthesis of sub-barcode molecule library
acgtggatagactcctcgac

SEQ ID NO: 45 - DNA, 20 bp, Artificial Sequence
  Sequence used in the synthesis of sub-barcode molecule library
actaggatagactcctcgac

SEQ ID NO: 46 - DNA, 20 bp, Artificial Sequence
  Sequence used in the synthesis of sub-barcode molecule library
actcggatagactcctcgac

SEQ ID NO: 47 - DNA, 20 bp, Artificial Sequence
  Sequence used in the synthesis of sub-barcode molecule library
actgggatagactcctcgac

SEQ ID NO: 48 - DNA, 20 bp, Artificial Sequence
  Sequence used in the synthesis of sub-barcode molecule library
acttggatagactcctcgac

SEQ ID NO: 49 - DNA, 20 bp, Artificial Sequence
  Sequence used in the synthesis of sub-barcode molecule library
agaaggatagactcctcgac

SEQ ID NO: 50 - DNA, 20 bp, Artificial Sequence
  Sequence used in the synthesis of sub-barcode molecule library
agacggatagactcctcgac

SEQ ID NO: 51 - DNA, 20 bp, Artificial Sequence
  Sequence used in the synthesis of sub-barcode molecule library
agagggatagactcctcgac

SEQ ID NO: 52 - DNA, 20 bp, Artificial Sequence
  Sequence used in the synthesis of sub-barcode molecule library
agatggatagactcctcgac

SEQ ID NO: 53 - DNA, 20 bp, Artificial Sequence
  Sequence used in the synthesis of sub-barcode molecule library
agcaggatagactcctcgac

SEQ ID NO: 54 - DNA, 20 bp, Artificial Sequence
  Sequence used in the synthesis of sub-barcode molecule library
agccggatagactcctcgac

SEQ ID NO: 55 - DNA, 20 bp, Artificial Sequence
  Sequence used in the synthesis of sub-barcode molecule library
agcgggatagactcctcgac

SEQ ID NO: 56 - DNA, 20 bp, Artificial Sequence
  Sequence used in the synthesis of sub-barcode molecule library
agctggatagactcctcgac

SEQ ID NO: 57 - DNA, 20 bp, Artificial Sequence
  Sequence used in the synthesis of sub-barcode molecule library
aggaggatagactcctcgac

SEQ ID NO: 58 - DNA, 20 bp, Artificial Sequence
  Sequence used in the synthesis of sub-barcode molecule library
aggcggatagactcctcgac

SEQ ID NO: 59 - DNA, 20 bp, Artificial Sequence
  Sequence used in the synthesis of sub-barcode molecule library
agggggatagactcctcgac

SEQ ID NO: 60 - DNA, 20 bp, Artificial Sequence
  Sequence used in the synthesis of sub-barcode molecule library
aggtggatagactcctcgac

SEQ ID NO: 61 - DNA, 20 bp, Artificial Sequence
  Sequence used in the synthesis of sub-barcode molecule library
agtaggatagactcctcgac

SEQ ID NO: 62 - DNA, 20 bp, Artificial Sequence
  Sequence used in the synthesis of sub-barcode molecule library
agtcggatagactcctcgac

SEQ ID NO: 63 - DNA, 20 bp, Artificial Sequence
  Sequence used in the synthesis of sub-barcode molecule library
agtgggatagactcctcgac

SEQ ID NO: 64 - DNA, 20 bp, Artificial Sequence
  Sequence used in the synthesis of sub-barcode molecule library
agttggatagactcctcgac

SEQ ID NO: 65 - DNA, 20 bp, Artificial Sequence
  Sequence used in the synthesis of sub-barcode molecule library
ataaggatagactcctcgac

SEQ ID NO: 66 - DNA, 20 bp, Artificial Sequence
  Sequence used in the synthesis of sub-barcode molecule library
atacggatagactcctcgac

SEQ ID NO: 67 - DNA, 20 bp, Artificial Sequence
  Sequence used in the synthesis of sub-barcode molecule library
atagggatagactcctcgac

SEQ ID NO: 68 - DNA, 20 bp, Artificial Sequence
  Sequence used in the synthesis of sub-barcode molecule library
atatggatagactcctcgac

SEQ ID NO: 69 - DNA, 20 bp, Artificial Sequence
  Sequence used in the synthesis of sub-barcode molecule library
atcaggatagactcctcgac

SEQ ID NO: 70 - DNA, 20 bp, Artificial Sequence
  Sequence used in the synthesis of sub-barcode molecule library
atccggatagactcctcgac

SEQ ID NO: 71 - DNA, 20 bp, Artificial Sequence
  Sequence used in the synthesis of sub-barcode molecule library
atcgggatagactcctcgac

SEQ ID NO: 72 - DNA, 20 bp, Artificial Sequence
  Sequence used in the synthesis of sub-barcode molecule library
atctggatagactcctcgac

SEQ ID NO: 73 - DNA, 20 bp, Artificial Sequence
  Sequence used in the synthesis of sub-barcode molecule library
atgaggatagactcctcgac

SEQ ID NO: 74 - DNA, 20 bp, Artificial Sequence
  Sequence used in the synthesis of sub-barcode molecule library
atgcggatagactcctcgac

SEQ ID NO: 75 - DNA, 20 bp, Artificial Sequence
  Sequence used in the synthesis of sub-barcode molecule library
atggggatagactcctcgac

SEQ ID NO: 76 - DNA, 20 bp, Artificial Sequence
  Sequence used in the synthesis of sub-barcode molecule library
atgtggatagactcctcgac

SEQ ID NO: 77 - DNA, 20 bp, Artificial Sequence
  Sequence used in the synthesis of sub-barcode molecule library
attaggatagactcctcgac

SEQ ID NO: 78 - DNA, 20 bp, Artificial Sequence
  Sequence used in the synthesis of sub-barcode molecule library
attcggatagactcctcgac

SEQ ID NO: 79 - DNA, 20 bp, Artificial Sequence
  Sequence used in the synthesis of sub-barcode molecule library
attgggatagactcctcgac

SEQ ID NO: 80 - DNA, 20 bp, Artificial Sequence
  Sequence used in the synthesis of sub-barcode molecule library
atttggatagactcctcgac

SEQ ID NO: 81 - DNA, 20 bp, Artificial Sequence
  Sequence used in the synthesis of sub-barcode molecule library
caaaggatagactcctcgac

SEQ ID NO: 82 - DNA, 20 bp, Artificial Sequence
  Sequence used in the synthesis of sub-barcode molecule library
caacggatagactcctcgac

SEQ ID NO: 83 - DNA, 20 bp, Artificial Sequence
  Sequence used in the synthesis of sub-barcode molecule library
caagggatagactcctcgac

SEQ ID NO: 84 - DNA, 20 bp, Artificial Sequence
  Sequence used in the synthesis of sub-barcode molecule library
caatggatagactcctcgac

SEQ ID NO: 85 - DNA, 20 bp, Artificial Sequence
  Sequence used in the synthesis of sub-barcode molecule library
cacaggatagactcctcgac

SEQ ID NO: 86 - DNA, 20 bp, Artificial Sequence
  Sequence used in the synthesis of sub-barcode molecule library
caccggatagactcctcgac

SEQ ID NO: 87 - DNA, 20 bp, Artificial Sequence
  Sequence used in the synthesis of sub-barcode molecule library
cacgggatagactcctcgac

SEQ ID NO: 88 - DNA, 20 bp, Artificial Sequence
  Sequence used in the synthesis of sub-barcode molecule library
cactggatagactcctcgac

SEQ ID NO: 89 - DNA, 20 bp, Artificial Sequence
  Sequence used in the synthesis of sub-barcode molecule library
cagaggatagactcctcgac

SEQ ID NO: 90 - DNA, 20 bp, Artificial Sequence
  Sequence used in the synthesis of sub-barcode molecule library
cagcggatagactcctcgac

SEQ ID NO: 91 - DNA, 20 bp, Artificial Sequence
  Sequence used in the synthesis of sub-barcode molecule library
caggggatagactcctcgac

SEQ ID NO: 92 - DNA, 20 bp, Artificial Sequence
  Sequence used in the synthesis of sub-barcode molecule library
cagtggatagactcctcgac

SEQ ID NO: 93 - DNA, 20 bp, Artificial Sequence
  Sequence used in the synthesis of sub-barcode molecule library
cataggatagactcctcgac

SEQ ID NO: 94 - DNA, 20 bp, Artificial Sequence
  Sequence used in the synthesis of sub-barcode molecule library
catcggatagactcctcgac

SEQ ID NO: 95 - DNA, 20 bp, Artificial Sequence
  Sequence used in the synthesis of sub-barcode molecule library
catgggatagactcctcgac

SEQ ID NO: 96 - DNA, 20 bp, Artificial Sequence
  Sequence used in the synthesis of sub-barcode molecule library
cattggatagactcctcgac

SEQ ID NO: 97 - DNA, 20 bp, Artificial Sequence
  Sequence used in the synthesis of sub-barcode molecule library
ccaaggatagactcctcgac

SEQ ID NO: 98 - DNA, 20 bp, Artificial Sequence
  Sequence used in the synthesis of sub-barcode molecule library
ccacggatagactcctcgac

SEQ ID NO: 99 - DNA, 20 bp, Artificial Sequence
  Sequence used in the synthesis of sub-barcode molecule library
ccagggatagactcctcgac

SEQ ID NO: 100 - DNA, 20 bp, Artificial Sequence
  Sequence used in the synthesis of sub-barcode molecule library
ccatggatagactcctcgac

SEQ ID NO: 101 - DNA, 20 bp, Artificial Sequence
  Sequence used in the synthesis of sub-barcode molecule library
cccaggatagactcctcgac

SEQ ID NO: 102 - DNA, 20 bp, Artificial Sequence
  Sequence used in the synthesis of sub-barcode molecule library
cccgggatagactcctcgac

SEQ ID NO: 103 - DNA, 20 bp, Artificial Sequence
  Sequence used in the synthesis of sub-barcode molecule library
ccctggatagactcctcgac

SEQ ID NO: 104 - DNA, 20 bp, Artificial Sequence
  Sequence used in the synthesis of sub-barcode molecule library
ccgaggatagactcctcgac

SEQ ID NO: 105 - DNA, 20 bp, Artificial Sequence
  Sequence used in the synthesis of sub-barcode molecule library
ccgcggatagactcctcgac

SEQ ID NO: 106 - DNA, 20 bp, Artificial Sequence
  Sequence used in the synthesis of sub-barcode molecule library
ccggggatagactcctcgac

SEQ ID NO: 107 - DNA, 20 bp, Artificial Sequence
  Sequence used in the synthesis of sub-barcode molecule library
ccgtggatagactcctcgac

SEQ ID NO: 108 - DNA, 20 bp, Artificial Sequence
  Sequence used in the synthesis of sub-barcode molecule library
cctaggatagactcctcgac

SEQ ID NO: 109 - DNA, 20 bp, Artificial Sequence
  Sequence used in the synthesis of sub-barcode molecule library
cctcggatagactcctcgac

SEQ ID NO: 110 - DNA, 20 bp, Artificial Sequence
  Sequence used in the synthesis of sub-barcode molecule library
cctgggatagactcctcgac

SEQ ID NO: 111 - DNA, 20 bp, Artificial Sequence
  Sequence used in the synthesis of sub-barcode molecule library
ccttggatagactcctcgac

SEQ ID NO: 112 - DNA, 20 bp, Artificial Sequence
  Sequence used in the synthesis of sub-barcode molecule library
cgaaggatagactcctcgac

SEQ ID NO: 113 - DNA, 20 bp, Artificial Sequence
  Sequence used in the synthesis of sub-barcode molecule library
cgacggatagactcctcgac

SEQ ID NO: 114 - DNA, 20 bp, Artificial Sequence
  Sequence used in the synthesis of sub-barcode molecule library
cgagggatagactcctcgac

SEQ ID NO: 115 - DNA, 20 bp, Artificial Sequence
  Sequence used in the synthesis of sub-barcode molecule library
cgatggatagactcctcgac

SEQ ID NO: 116 - DNA, 20 bp, Artificial Sequence
  Sequence used in the synthesis of sub-barcode molecule library
cgcaggatagactcctcgac

SEQ ID NO: 117 - DNA, 20 bp, Artificial Sequence
  Sequence used in the synthesis of sub-barcode molecule library
cgccggatagactcctcgac

SEQ ID NO: 118 - DNA, 20 bp, Artificial Sequence
  Sequence used in the synthesis of sub-barcode molecule library
cgcgggatagactcctcgac

SEQ ID NO: 119 - DNA, 20 bp, Artificial Sequence
  Sequence used in the synthesis of sub-barcode molecule library
cgctggatagactcctcgac

SEQ ID NO: 120 - DNA, 20 bp, Artificial Sequence
  Sequence used in the synthesis of sub-barcode molecule library
cggaggatagactcctcgac

SEQ ID NO: 121 - DNA, 20 bp, Artificial Sequence
  Sequence used in the synthesis of sub-barcode molecule library
cggcggatagactcctcgac

SEQ ID NO: 122 - DNA, 20 bp, Artificial Sequence
  Sequence used in the synthesis of sub-barcode molecule library
cgggggatagactcctcgac

SEQ ID NO: 123 - DNA, 20 bp, Artificial Sequence
  Sequence used in the synthesis of sub-barcode molecule library
cggtggatagactcctcgac

SEQ ID NO: 124 - DNA, 20 bp, Artificial Sequence
  Sequence used in the synthesis of sub-barcode molecule library
cgtaggatagactcctcgac

SEQ ID NO: 125 - DNA, 20 bp, Artificial Sequence
  Sequence used in the synthesis of sub-barcode molecule library
cgtcggatagactcctcgac

SEQ ID NO: 126 - DNA, 20 bp, Artificial Sequence
  Sequence used in the synthesis of sub-barcode molecule library
cgtgggatagactcctcgac

SEQ ID NO: 127 - DNA, 20 bp, Artificial Sequence
  Sequence used in the synthesis of sub-barcode molecule library
cgttggatagactcctcgac

SEQ ID NO: 128 - DNA, 20 bp, Artificial Sequence
  Sequence used in the synthesis of sub-barcode molecule library
ctaaggatagactcctcgac

SEQ ID NO: 129 - DNA, 20 bp, Artificial Sequence
  Sequence used in the synthesis of sub-barcode molecule library
ctacggatagactcctcgac

SEQ ID NO: 130 - DNA, 20 bp, Artificial Sequence
  Sequence used in the synthesis of sub-barcode molecule library
ctagggatagactcctcgac

SEQ ID NO: 131 - DNA, 20 bp, Artificial Sequence
  Sequence used in the synthesis of sub-barcode molecule library
ctatggatagactcctcgac

SEQ ID NO: 132 - DNA, 20 bp, Artificial Sequence
  Sequence used in the synthesis of sub-barcode molecule library
ctcaggatagactcctcgac

SEQ ID NO: 133 - DNA, 20 bp, Artificial Sequence
  Sequence used in the synthesis of sub-barcode molecule library
ctccggatagactcctcgac

SEQ ID NO: 134 - DNA, 20 bp, Artificial Sequence
  Sequence used in the synthesis of sub-barcode molecule library
ctcgggatagactcctcgac

SEQ ID NO: 135 - DNA, 20 bp, Artificial Sequence
  Sequence used in the synthesis of sub-barcode molecule library
ctctggatagactcctcgac

SEQ ID NO: 136 - DNA, 20 bp, Artificial Sequence
  Sequence used in the synthesis of sub-barcode molecule library
ctgaggatagactcctcgac

SEQ ID NO: 137 - DNA, 20 bp, Artificial Sequence
  Sequence used in the synthesis of sub-barcode molecule library
ctgcggatagactcctcgac

SEQ ID NO: 138 - DNA, 20 bp, Artificial Sequence
  Sequence used in the synthesis of sub-barcode molecule library
ctggggatagactcctcgac

SEQ ID NO: 139 - DNA, 20 bp, Artificial Sequence
  Sequence used in the synthesis of sub-barcode molecule library
ctgtggatagactcctcgac

SEQ ID NO: 140 - DNA, 20 bp, Artificial Sequence
  Sequence used in the synthesis of sub-barcode molecule library
cttaggatagactcctcgac

SEQ ID NO: 141 - DNA, 20 bp, Artificial Sequence
  Sequence used in the synthesis of sub-barcode molecule library
cttcggatagactcctcgac

SEQ ID NO: 142 - DNA, 20 bp, Artificial Sequence
  Sequence used in the synthesis of sub-barcode molecule library
cttgggatagactcctcgac

SEQ ID NO: 143 - DNA, 20 bp, Artificial Sequence
  Sequence used in the synthesis of sub-barcode molecule library
ctttggatagactcctcgac

SEQ ID NO: 144 - DNA, 20 bp, Artificial Sequence
  Sequence used in the synthesis of sub-barcode molecule library
gaaaggatagactcctcgac

SEQ ID NO: 145 - DNA, 20 bp, Artificial Sequence
  Sequence used in the synthesis of sub-barcode molecule library
gaacggatagactcctcgac

SEQ ID NO: 146 - DNA, 20 bp, Artificial Sequence
  Sequence used in the synthesis of sub-barcode molecule library
gaagggatagactcctcgac

SEQ ID NO: 147 - DNA, 20 bp, Artificial Sequence
  Sequence used in the synthesis of sub-barcode molecule library
gaatggatagactcctcgac

SEQ ID NO: 148 - DNA, 20 bp, Artificial Sequence
  Sequence used in the synthesis of sub-barcode molecule library
gacaggatagactcctcgac

SEQ ID NO: 149 - DNA, 20 bp, Artificial Sequence
  Sequence used in the synthesis of sub-barcode molecule library
gaccggatagactcctcgac

SEQ ID NO: 150 - DNA, 20 bp, Artificial Sequence
  Sequence used in the synthesis of sub-barcode molecule library
gacgggatagactcctcgac

SEQ ID NO: 151 - DNA, 20 bp, Artificial Sequence
  Sequence used in the synthesis of sub-barcode molecule library
gactggatagactcctcgac

SEQ ID NO: 152 - DNA, 20 bp, Artificial Sequence
  Sequence used in the synthesis of sub-barcode molecule library
gagaggatagactcctcgac

SEQ ID NO: 153 - DNA, 20 bp, Artificial Sequence
  Sequence used in the synthesis of sub-barcode molecule library
gagcggatagactcctcgac

SEQ ID NO: 154 - DNA, 20 bp, Artificial Sequence
  Sequence used in the synthesis of sub-barcode molecule library
gaggggatagactcctcgac

SEQ ID NO: 155 - DNA, 20 bp, Artificial Sequence
  Sequence used in the synthesis of sub-barcode molecule library
gagtggatagactcctcgac

SEQ ID NO: 156 - DNA, 20 bp, Artificial Sequence
  Sequence used in the synthesis of sub-barcode molecule library
gataggatagactcctcgac

SEQ ID NO: 157 - DNA, 20 bp, Artificial Sequence
  Sequence used in the synthesis of sub-barcode molecule library
gatcggatagactcctcgac

SEQ ID NO: 158 - DNA, 20 bp, Artificial Sequence
  Sequence used in the synthesis of sub-barcode molecule library
gatgggatagactcctcgac

SEQ ID NO: 159 - DNA, 20 bp, Artificial Sequence
  Sequence used in the synthesis of sub-barcode molecule library
gattggatagactcctcgac

SEQ ID NO: 160 - DNA, 20 bp, Artificial Sequence
  Sequence used in the synthesis of sub-barcode molecule library
gcaaggatagactcctcgac

SEQ ID NO: 161 - DNA, 20 bp, Artificial Sequence
  Sequence used in the synthesis of sub-barcode molecule library
gcacggatagactcctcgac

SEQ ID NO: 162 - DNA, 20 bp, Artificial Sequence
  Sequence used in the synthesis of sub-barcode molecule library
gcagggatagactcctcgac

SEQ ID NO: 163 - DNA, 20 bp, Artificial Sequence
  Sequence used in the synthesis of sub-barcode molecule library
gcatggatagactcctcgac

SEQ ID NO: 164 - DNA, 20 bp, Artificial Sequence
  Sequence used in the synthesis of sub-barcode molecule library
gccaggatagactcctcgac

SEQ ID NO: 165 - DNA, 20 bp, Artificial Sequence
  Sequence used in the synthesis of sub-barcode molecule library
gcccggatagactcctcgac

SEQ ID NO: 166 - DNA, 20 bp, Artificial Sequence
  Sequence used in the synthesis of sub-barcode molecule library
gccgggatagactcctcgac

SEQ ID NO: 167 - DNA, 20 bp, Artificial Sequence
  Sequence used in the synthesis of sub-barcode molecule library
gcctggatagactcctcgac

SEQ ID NO: 168 - DNA, 20 bp, Artificial Sequence
  Sequence used in the synthesis of sub-barcode molecule library
gcgaggatagactcctcgac

SEQ ID NO: 169 - DNA, 20 bp, Artificial Sequence
  Sequence used in the synthesis of sub-barcode molecule library
gcgcggatagactcctcgac

SEQ ID NO: 170 - DNA, 20 bp, Artificial Sequence
  Sequence used in the synthesis of sub-barcode molecule library
gcggggatagactcctcgac

SEQ ID NO: 171 - DNA, 20 bp, Artificial Sequence
  Sequence used in the synthesis of sub-barcode molecule library
gcgtggatagactcctcgac

SEQ ID NO: 172 - DNA, 20 bp, Artificial Sequence
  Sequence used in the synthesis of sub-barcode molecule library
gctaggatagactcctcgac

SEQ ID NO: 173 - DNA, 20 bp, Artificial Sequence
  Sequence used in the synthesis of sub-barcode molecule library
gctcggatagactcctcgac

SEQ ID NO: 174 - DNA, 20 bp, Artificial Sequence
  Sequence used in the synthesis of sub-barcode molecule library
gctgggatagactcctcgac

SEQ ID NO: 175 - DNA, 20 bp, Artificial Sequence
  Sequence used in the synthesis of sub-barcode molecule library
gcttggatagactcctcgac

SEQ ID NO: 176 - DNA, 20 bp, Artificial Sequence
  Sequence used in the synthesis of sub-barcode molecule library
ggaaggatagactcctcgac

SEQ ID NO: 177 - DNA, 20 bp, Artificial Sequence
  Sequence used in the synthesis of sub-barcode molecule library
ggacggatagactcctcgac

SEQ ID NO: 178 - DNA, 20 bp, Artificial Sequence
  Sequence used in the synthesis of sub-barcode molecule library
ggagggatagactcctcgac

SEQ ID NO: 179 - DNA, 20 bp, Artificial Sequence
  Sequence used in the synthesis of sub-barcode molecule library
ggatggatagactcctcgac

SEQ ID NO: 180 - DNA, 20 bp, Artificial Sequence
  Sequence used in the synthesis of sub-barcode molecule library
ggcaggatagactcctcgac

SEQ ID NO: 181 - DNA, 20 bp, Artificial Sequence
  Sequence used in the synthesis of sub-barcode molecule library
ggccggatagactcctcgac

SEQ ID NO: 182 - DNA, 20 bp, Artificial Sequence
  Sequence used in the synthesis of sub-barcode molecule library
ggcgggatagactcctcgac

SEQ ID NO: 183 - DNA, 20 bp, Artificial Sequence
  Sequence used in the synthesis of sub-barcode molecule library
ggctggatagactcctcgac

SEQ ID NO: 184 - DNA, 20 bp, Artificial Sequence
  Sequence used in the synthesis of sub-barcode molecule library
gggaggatagactcctcgac

SEQ ID NO: 185 - DNA, 20 bp, Artificial Sequence
  Sequence used in the synthesis of sub-barcode molecule library
gggcggatagactcctcgac

SEQ ID NO: 186 - DNA, 20 bp, Artificial Sequence
  Sequence used in the synthesis of sub-barcode molecule library
gggtggatagactcctcgac

SEQ ID NO: 187 - DNA, 20 bp, Artificial Sequence
  Sequence used in the synthesis of sub-barcode molecule library
ggtaggatagactcctcgac

SEQ ID NO: 188 - DNA, 20 bp, Artificial Sequence
  Sequence used in the synthesis of sub-barcode molecule library
ggtcggatagactcctcgac

SEQ ID NO: 189 - DNA, 20 bp, Artificial Sequence
  Sequence used in the synthesis of sub-barcode molecule library
ggtgggatagactcctcgac

SEQ ID NO: 190 - DNA, 20 bp, Artificial Sequence
  Sequence used in the synthesis of sub-barcode molecule library
ggttggatagactcctcgac

SEQ ID NO: 191 - DNA, 20 bp, Artificial Sequence
  Sequence used in the synthesis of sub-barcode molecule library
gtaaggatagactcctcgac

SEQ ID NO: 192 - DNA, 20 bp, Artificial Sequence
  Sequence used in the synthesis of sub-barcode molecule library
gtacggatagactcctcgac

SEQ ID NO: 193 - DNA, 20 bp, Artificial Sequence
  Sequence used in the synthesis of sub-barcode molecule library
gtagggatagactcctcgac

SEQ ID NO: 194 - DNA, 20 bp, Artificial Sequence
  Sequence used in the synthesis of sub-barcode molecule library
gtatggatagactcctcgac

SEQ ID NO: 195 - DNA, 20 bp, Artificial Sequence
  Sequence used in the synthesis of sub-barcode molecule library
gtcaggatagactcctcgac

SEQ ID NO: 196 - DNA, 20 bp, Artificial Sequence
  Sequence used in the synthesis of sub-barcode molecule library
gtccggatagactcctcgac

SEQ ID NO: 197 - DNA, 20 bp, Artificial Sequence
  Sequence used in the synthesis of sub-barcode molecule library
gtcgggatagactcctcgac

SEQ ID NO: 198 - DNA, 20 bp, Artificial Sequence
  Sequence used in the synthesis of sub-barcode molecule library
gtctggatagactcctcgac

SEQ ID NO: 199 - DNA, 20 bp, Artificial Sequence
  Sequence used in the synthesis of sub-barcode molecule library
gtgaggatagactcctcgac

SEQ ID NO: 200 - DNA, 20 bp, Artificial Sequence
  Sequence used in the synthesis of sub-barcode molecule library
gtgcggatagactcctcgac

SEQ ID NO: 201 - DNA, 20 bp, Artificial Sequence
  Sequence used in the synthesis of sub-barcode molecule library
gtggggatagactcctcgac

SEQ ID NO: 202 - DNA, 20 bp, Artificial Sequence
  Sequence used in the synthesis of sub-barcode molecule library
gtgtggatagactcctcgac

SEQ ID NO: 203 - DNA, 20 bp, Artificial Sequence
  Sequence used in the synthesis of sub-barcode molecule library
gttaggatagactcctcgac

SEQ ID NO: 204 - DNA, 20 bp, Artificial Sequence
  Sequence used in the synthesis of sub-barcode molecule library
gttcggatagactcctcgac

SEQ ID NO: 205 - DNA, 20 bp, Artificial Sequence
  Sequence used in the synthesis of sub-barcode molecule library
gttgggatagactcctcgac

SEQ ID NO: 206 - DNA, 20 bp, Artificial Sequence
  Sequence used in the synthesis of sub-barcode molecule library
gtttggatagactcctcgac

SEQ ID NO: 207 - DNA, 20 bp, Artificial Sequence
  Sequence used in the synthesis of sub-barcode molecule library
taaaggatagactcctcgac

SEQ ID NO: 208 - DNA, 20 bp, Artificial Sequence
  Sequence used in the synthesis of sub-barcode molecule library
taacggatagactcctcgac

SEQ ID NO: 209 - DNA, 20 bp, Artificial Sequence
  Sequence used in the synthesis of sub-barcode molecule library
taagggatagactcctcgac

SEQ ID NO: 210 - DNA, 20 bp, Artificial Sequence
  Sequence used in the synthesis of sub-barcode molecule library
taatggatagactcctcgac

SEQ ID NO: 211 - DNA, 20 bp, Artificial Sequence
  Sequence used in the synthesis of sub-barcode molecule library
tacaggatagactcctcgac

SEQ ID NO: 212 - DNA, 20 bp, Artificial Sequence
  Sequence used in the synthesis of sub-barcode molecule library
taccggatagactcctcgac

SEQ ID NO: 213 - DNA, 20 bp, Artificial Sequence
  Sequence used in the synthesis of sub-barcode molecule library
tacgggatagactcctcgac

SEQ ID NO: 214 - DNA, 20 bp, Artificial Sequence
  Sequence used in the synthesis of sub-barcode molecule library
tactggatagactcctcgac

SEQ ID NO: 215 - DNA, 20 bp, Artificial Sequence
  Sequence used in the synthesis of sub-barcode molecule library
tagaggatagactcctcgac

SEQ ID NO: 216 - DNA, 20 bp, Artificial Sequence
  Sequence used in the synthesis of sub-barcode molecule library
tagcggatagactcctcgac

SEQ ID NO: 217 - DNA, 20 bp, Artificial Sequence
  Sequence used in the synthesis of sub-barcode molecule library
taggggatagactcctcgac

SEQ ID NO: 218 - DNA, 20 bp, Artificial Sequence
  Sequence used in the synthesis of sub-barcode molecule library
tagtggatagactcctcgac

SEQ ID NO: 219 - DNA, 20 bp, Artificial Sequence
  Sequence used in the synthesis of sub-barcode molecule library
tataggatagactcctcgac

SEQ ID NO: 220 - DNA, 20 bp, Artificial Sequence
  Sequence used in the synthesis of sub-barcode molecule library
tatcggatagactcctcgac

SEQ ID NO: 221 - DNA, 20 bp, Artificial Sequence
  Sequence used in the synthesis of sub-barcode molecule library
tatgggatagactcctcgac

SEQ ID NO: 222 - DNA, 20 bp, Artificial Sequence
  Sequence used in the synthesis of sub-barcode molecule library
tattggatagactcctcgac

SEQ ID NO: 223 - DNA, 20 bp, Artificial Sequence
  Sequence used in the synthesis of sub-barcode molecule library
tcaaggatagactcctcgac

SEQ ID NO: 224 - DNA, 20 bp, Artificial Sequence
  Sequence used in the synthesis of sub-barcode molecule library
tcacggatagactcctcgac

SEQ ID NO: 225 - DNA, 20 bp, Artificial Sequence
  Sequence used in the synthesis of sub-barcode molecule library
tcagggatagactcctcgac

SEQ ID NO: 226 - DNA, 20 bp, Artificial Sequence
  Sequence used in the synthesis of sub-barcode molecule library
tcatggatagactcctcgac

SEQ ID NO: 227 - DNA, 20 bp, Artificial Sequence
  Sequence used in the synthesis of sub-barcode molecule library
tccaggatagactcctcgac

SEQ ID NO: 228 - DNA, 20 bp, Artificial Sequence
  Sequence used in the synthesis of sub-barcode molecule library
tcccggatagactcctcgac

SEQ ID NO: 229 - DNA, 20 bp, Artificial Sequence
  Sequence used in the synthesis of sub-barcode molecule library
tccgggatagactcctcgac

SEQ ID NO: 230 - DNA, 20 bp, Artificial Sequence
  Sequence used in the synthesis of sub-barcode molecule library
tcctggatagactcctcgac

SEQ ID NO: 231 - DNA, 20 bp, Artificial Sequence
  Sequence used in the synthesis of sub-barcode molecule library
tcgaggatagactcctcgac

SEQ ID NO: 232 - DNA, 20 bp, Artificial Sequence
  Sequence used in the synthesis of sub-barcode molecule library
tcgcggatagactcctcgac

SEQ ID NO: 233 - DNA, 20 bp, Artificial Sequence
  Sequence used in the synthesis of sub-barcode molecule library
tcggggatagactcctcgac

SEQ ID NO: 234 - DNA, 20 bp, Artificial Sequence
  Sequence used in the synthesis of sub-barcode molecule library
tcgtggatagactcctcgac

SEQ ID NO: 235 - DNA, 20 bp, Artificial Sequence
  Sequence used in the synthesis of sub-barcode molecule library
tctaggatagactcctcgac

SEQ ID NO: 236 - DNA, 20 bp, Artificial Sequence
  Sequence used in the synthesis of sub-barcode molecule library
tctcggatagactcctcgac

SEQ ID NO: 237 - DNA, 20 bp, Artificial Sequence
  Sequence used in the synthesis of sub-barcode molecule library
tctgggatagactcctcgac

SEQ ID NO: 238 - DNA, 20 bp, Artificial Sequence
  Sequence used in the synthesis of sub-barcode molecule library
tcttggatagactcctcgac

SEQ ID NO: 239 - DNA, 20 bp, Artificial Sequence
  Sequence used in the synthesis of sub-barcode molecule library
tgaaggatagactcctcgac

SEQ ID NO: 240 - DNA, 20 bp, Artificial Sequence
  Sequence used in the synthesis of sub-barcode molecule library
tgacggatagactcctcgac

SEQ ID NO: 241 - DNA, 20 bp, Artificial Sequence
  Sequence used in the synthesis of sub-barcode molecule library
tgagggatagactcctcgac

SEQ ID NO: 242 - DNA, 20 bp, Artificial Sequence
  Sequence used in the synthesis of sub-barcode molecule library
tgatggatagactcctcgac

SEQ ID NO: 243 - DNA, 20 bp, Artificial Sequence
  Sequence used in the synthesis of sub-barcode molecule library
tgcaggatagactcctcgac

SEQ ID NO: 244 - DNA, 20 bp, Artificial Sequence
  Sequence used in the synthesis of sub-barcode molecule library
tgccggatagactcctcgac

SEQ ID NO: 245 - DNA, 20 bp, Artificial Sequence
  Sequence used in the synthesis of sub-barcode molecule library
tgcgggatagactcctcgac

SEQ ID NO: 246 - DNA, 20 bp, Artificial Sequence
  Sequence used in the synthesis of sub-barcode molecule library
tgctggatagactcctcgac

SEQ ID NO: 247 - DNA, 20 bp, Artificial Sequence
  Sequence used in the synthesis of sub-barcode molecule library
tggaggatagactcctcgac

SEQ ID NO: 248 - DNA, 20 bp, Artificial Sequence
  Sequence used in the synthesis of sub-barcode molecule library
tggcggatagactcctcgac

SEQ ID NO: 249 - DNA, 20 bp, Artificial Sequence
  Sequence used in the synthesis of sub-barcode molecule library
tgggggatagactcctcgac

SEQ ID NO: 250 - DNA, 20 bp, Artificial Sequence
  Sequence used in the synthesis of sub-barcode molecule library
tggtggatagactcctcgac

SEQ ID NO: 251 - DNA, 20 bp, Artificial Sequence
  Sequence used in the synthesis of sub-barcode molecule library
tgtaggatagactcctcgac

SEQ ID NO: 252 - DNA, 20 bp, Artificial Sequence
  Sequence used in the synthesis of sub-barcode molecule library
tgtcggatagactcctcgac

SEQ ID NO: 253 - DNA, 20 bp, Artificial Sequence
  Sequence used in the synthesis of sub-barcode molecule library
tgtgggatagactcctcgac

SEQ ID NO: 254 - DNA, 20 bp, Artificial Sequence
  Sequence used in the synthesis of sub-barcode molecule library
tgttggatagactcctcgac

SEQ ID NO: 255 - DNA, 20 bp, Artificial Sequence
  Sequence used in the synthesis of sub-barcode molecule library
ttaaggatagactcctcgac

SEQ ID NO: 256 - DNA, 20 bp, Artificial Sequence
  Sequence used in the synthesis of sub-barcode molecule library
ttacggatagactcctcgac

SEQ ID NO: 257 - DNA, 20 bp, Artificial Sequence
  Sequence used in the synthesis of sub-barcode molecule library
ttagggatagactcctcgac

SEQ ID NO: 258 - DNA, 20 bp, Artificial Sequence
  Sequence used in the synthesis of sub-barcode molecule library
ttatggatagactcctcgac

SEQ ID NO: 259 - DNA, 20 bp, Artificial Sequence
  Sequence used in the synthesis of sub-barcode molecule library
ttcaggatagactcctcgac

SEQ ID NO: 260 - DNA, 20 bp, Artificial Sequence
  Sequence used in the synthesis of sub-barcode molecule library
ttccggatagactcctcgac

SEQ ID NO: 261 - DNA, 20 bp, Artificial Sequence
  Sequence used in the synthesis of sub-barcode molecule library
ttcgggatagactcctcgac

SEQ ID NO: 262 - DNA, 20 bp, Artificial Sequence
  Sequence used in the synthesis of sub-barcode molecule library
ttctggatagactcctcgac

SEQ ID NO: 263 - DNA, 20 bp, Artificial Sequence
  Sequence used in the synthesis of sub-barcode molecule library
ttgaggatagactcctcgac

SEQ ID NO: 264 - DNA, 20 bp, Artificial Sequence
  Sequence used in the synthesis of sub-barcode molecule library
ttgcggatagactcctcgac

SEQ ID NO: 265 - DNA, 20 bp, Artificial Sequence
  Sequence used in the synthesis of sub-barcode molecule library
ttggggatagactcctcgac

SEQ ID NO: 266 - DNA, 20 bp, Artificial Sequence
  Sequence used in the synthesis of sub-barcode molecule library
ttgtggatagactcctcgac

SEQ ID NO: 267 - DNA, 20 bp, Artificial Sequence
  Sequence used in the synthesis of sub-barcode molecule library
tttaggatagactcctcgac

SEQ ID NO: 268 - DNA, 20 bp, Artificial Sequence
  Sequence used in the synthesis of sub-barcode molecule library
tttcggatagactcctcgac

SEQ ID NO: 269 - DNA, 20 bp, Artificial Sequence
  Sequence used in the synthesis of sub-barcode molecule library
tttgggatagactcctcgac

SEQ ID NO: 270 - DNA, 47 bp, Artificial Sequence
  Primer
taatacgactcactatagggagataggacgatacgagtgtgtactcg

SEQ ID NO: 271 - DNA, 31 bp, Artificial Sequence
  Primer
ctgtcaaggtagactagcatgctcccatacg

SEQ ID NO: 272 - DNA, 24 bp, Artificial Sequence
  Primer
ctgtcaaggtagactagcatgctc

SEQ ID NO: 273 - DNA, 60 bp, Artificial Sequence
  Adaptor oligonucleotide
cctgactgctcgtcagttgattaagtactctgtgagatgatgatcagtagagcgagtcgt

SEQ ID NO: 274 - DNA, 50 bp, Artificial Sequence
  Primer
caccgagatctacactctttccctacacgacgctcttccgatcttgacct

SEQ ID NO: 275 - DNA, 59 bp, Artificial Sequence
  Synthetic template
  misc_feature (22)..(39): n is a, c, g, or t
atgatcagtagagcgagtcgtnnnnnnnnnnnnnnnnnntgctacgacttccgagtcca

SEQ ID NO: 276 - DNA, 27 bp, Artificial Sequence
  Primer
gctctactgatcattggactcggaagt

SEQ ID NO: 277 - DNA, 28 bp, Artificial Sequence
  Primer
tccgatcttggactcggaagtcgtagca

SEQ ID NO: 278 - DNA, 39 bp, Artificial Sequence; identical to SEQ ID NO: 17
  Primer

SEQ ID NO: 279 - DNA, 59 bp, Artificial Sequence
  BRCA1 adaptor oligonucleotide
cctgactgctcgtcagttgattaagtactctgtgagatgcttggcccctcttcggtaac

SEQ ID NO: 280 - DNA, 60 bp, Artificial Sequence
  BRCA1 adaptor oligonucleotide
cctgactgctcgtcagttgattaagtactctgtgagatgctgggagctcaaaagatggct

SEQ ID NO: 281 - DNA, 58 bp, Artificial Sequence
  BRCA1 adaptor oligonucleotide
cctgactgctcgtcagttgattaagtactctgtgagatgcagctgggctcaaaggacc

SEQ ID NO: 282 - DNA, 60 bp, Artificial Sequence
  BRCA1 adaptor oligonucleotide
cctgactgctcgtcagttgattaagtactctgtgagatgcagacaaattccccagcaggt

SEQ ID NO: 283 - DNA, 58 bp, Artificial Sequence
  BRCA1 adaptor oligonucleotide
cctgactgctcgtcagttgattaagtactctgtgagatgcatggtgtgaacccgggag

SEQ ID NO: 284 - DNA, 60 bp, Artificial Sequence
  BRCA1 adaptor oligonucleotide
cctgactgctcgtcagttgattaagtactctgtgagatgcccaaatcccaagtcgtgtgt

SEQ ID NO: 285 - DNA, 60 bp, Artificial Sequence
  BRCA1 adaptor oligonucleotide
cctgactgctcgtcagttgattaagtactctgtgagatgctcatccctggttccttgagg

SEQ ID NO: 286 - DNA, 60 bp, Artificial Sequence
  HLA-A adaptor oligonucleotide
cctgactgctcgtcagttgattaagtactctgtgaaaacggcctctgtggggagaagcaa

SEQ ID NO: 287 - DNA, 59 bp, Artificial Sequence
  HLA-A adaptor oligonucleotide
cctgactgctcgtcagttgattaagtactctgtgagatgcactgggctgaccgtggggt

SEQ ID NO: 288 - DNA, 60 bp, Artificial Sequence
  HLA-A adaptor oligonucleotide
cctgactgctcgtcagttgattaagtactctgcctgaatgwtctgactcttcccgtmaga

SEQ ID NO: 289 - DNA, 60 bp, Artificial Sequence
  DQB1 adaptor oligonucleotide
cctgactgctcgtcagttgattaagtactctgggatccccgcagaggatttcgtgtacca

SEQ ID NO: 290 - DNA, 60 bp, Artificial Sequence
  DQB1 adaptor oligonucleotide
cctgactgctcgtcagttgattaagtactctgtgagatggagcccacagtgaccatctcc

SEQ ID NO: 291 - DNA, 60 bp, Artificial Sequence
  BRCA1 reverse primer
cggtctcggcattcctgctgaaccgctcttccgatctgttctgagacacctgatgacctg

SEQ ID NO: 292 - DNA, 57 bp, Artificial Sequence
  BRCA1 reverse primer
cggtctcggcattcctgctgaaccgctcttccgatcttgaacccaggagtttgaggc

SEQ ID NO: 293 - DNA, 60 bp, Artificial Sequence
  BRCA1 reverse primer
cggtctcggcattcctgctgaaccgctcttccgatcttggagctttatctgctctgtgat

SEQ ID NO: 294 - DNA, 57 bp, Artificial Sequence
  BRCA1 reverse primer
cggtctcggcattcctgctgaaccgctcttccgatctttcactgtgatggccaggat

SEQ ID NO: 295 - DNA, 57 bp, Artificial Sequence
  BRCA1 reverse primer
cggtctcggcattcctgctgaaccgctcttccgatcttgacccaagcaagcctaaag

SEQ ID NO: 296 - DNA, 57 bp, Artificial Sequence
  BRCA1 reverse primer
cggtctcggcattcctgctgaaccgctcttccgatcttgccacagtagatgctcagt

SEQ ID NO: 297 - DNA, 58 bp, Artificial Sequence
  BRCA1 reverse primer
cggtctcggcattcctgctgaaccgctcttccgatctcccagcaaccatttcatttca

SEQ ID NO: 298 - DNA, 60 bp, Artificial Sequence
  HLA-A reverse primer
cggtctcggcattcctgctgaaccgctcttccgatcttggatctcggacccggagactgt

SEQ ID NO: 299 - DNA, 58 bp, Artificial Sequence
  HLA-A reverse primer
cggtctcggcattcctgctgaaccgctcttccgatctccctggtaccvgtgcgctgca

SEQ ID NO: 300 - DNA, 60 bp, Artificial Sequence
  HLA-A reverse primer
cggtctcggcattcctgctgaaccgctcttccgatctgaccctgctaaaggtctccagag

SEQ ID NO: 301 - DNA, 57 bp, Artificial Sequence
  HLA-A reverse primer
cggtctcggcattcctgctgaaccgctcttccgatctgaccctgctaaaggtcagag

SEQ ID NO: 302 - DNA, 60 bp, Artificial Sequence
  DQB1 reverse primer
cggtctcggcattcctgctgaaccgctcttccgatctaggacgctcacctctccgctgca

SEQ ID NO: 303 - DNA, 57 bp, Artificial Sequence
  DQB1 reverse primer
cggtctcggcattcctgctgaaccgctcttccgatctctggggtgctccacgtggca